European Patent Application EP 4 424 820 A1, published September 4, 2024. Title: DESIGNED SYNZIP PROTEIN DOMAINS FOR GENERATING ARTIFICIAL NONRIBOSOMAL PEPTIDE SYNTHETASES AND HYBRIDS THEREOF. Applicant: Max-Planck-Gesellschaft zur, Förderung der Wissenschaften e.V., München. The sequence listing filed with the application follows.

SEQUENCE LISTING (415 sequences)

SEQ ID NO: 1 - protein, 47 aa, synthetic construct
NLVAQLENEVASLENENETLKKKNLHKKDLIAYLEKEIANLRKKIEE

SEQ ID NO: 2 - protein, 50 aa, synthetic construct
ARNAYLRKKIARLKKDNLQLERDEQNLEKIIANLRDEIARLENEVASHEQ

SEQ ID NO: 3 - protein, 42 aa, synthetic construct
NEVTTLENDAAFIENENAYLEKEIARLRKEKAALRNRLAHKK

SEQ ID NO: 4 - protein, 54 aa, synthetic construct
QKVAELKNRVAVKLNRNEQLKNKVEELKNRNAYLKNELATLENEVARLENDVAE

SEQ ID NO: 5 - protein, 44 aa, synthetic construct
NTVKELKNYIQELEERNAELKNLKEHLKFAKAELEFELAAHKFE

SEQ ID NO: 6 - protein, 54 aa, synthetic construct
QKVAQLKNRVAYKLKENAKLENIVARLENDNANLEKDIANLEKDIANLERDVAR

SEQ ID NO: 7 - protein, 51 aa, synthetic construct
KEIEYLEKEIERLKDLREHLKQDNAAHRQELNALRLEEAKLEFILAHLLST

SEQ ID NO: 8 - protein, 51 aa, synthetic construct
KEIANLEKEIASLEKKVAVLKQRNAAHKQEVAALRKEIAYVEDEIQYVEDE

SEQ ID NO: 9 - protein, 36 aa, synthetic construct
QKVESLKQKIEELKQRKAQLKNDIANLEKEIAYAET

SEQ ID NO: 10 - protein, 42 aa, synthetic construct
NLLATLRSTAAVLENENHVLEKEKEKLRKEKEQLLNKLEAYK

SEQ ID NO: 11 - protein, 42 aa, synthetic construct
ELTDELKNKKEALRKDNAALLNELASLENEIANLEKEIAYFK

SEQ ID NO: 12 - protein, 42 aa, synthetic construct
NEDLVLENRLAALRNENAALENDLARLEKEIAYLEKEIEREK

SEQ ID NO: 13 - protein, 44 aa, synthetic construct
QKVEELKNKIAELENRNAVKKNRVAHLKQEIAYLKDELAAHEFE

SEQ ID NO: 14 - protein, 47 aa, synthetic construct
NDLDAYEREAEKLEKKNEVLRNRLAALENELATLRQEVASMKQELQS

SEQ ID NO: 15 - protein, 41 aa, synthetic construct
FENVTHEFILATLENENAKLRRLEAKLERELARLRNEVAWL

SEQ ID NO: 16 - protein, 42 aa, synthetic construct
NILASLENKKEELKKLNAHLLKEIENLEKEIANLEKEIAYFK

SEQ ID NO: 17 - protein, 42 aa, synthetic construct
NEKEELKSKKAELRNRIEQLKQKREQLKQKIANLRKEIEAYK

SEQ ID NO: 18 - protein, 41 aa, synthetic construct
SIAATLENDLARLENENARLEKDIANLERDLAKLEREEAYF

SEQ ID NO: 19 - protein, 45 aa, synthetic construct
NELESLENKKEELKNRNEELKQKREQLKQKLAALRNKLDAYKNRL

SEQ ID NO: 20 - protein, 44 aa, synthetic construct
STVEELLRAIQELEKRNAELKNRKEELKNLVAHLRQELAAHKYE

SEQ ID NO: 21 - protein, 42 aa, synthetic construct
NEVAQLENDVAVIENENAYLEKEIARLRKEIAALRDRLAHKK

SEQ ID NO: 22 - protein, 50 aa, synthetic construct
KRIAYLRKKIAALKKDNANLEKDIANLENEIERLIKEIKTLENEVASHEQ

SEQ ID NO: 23 - protein, 46 aa, synthetic construct
LVAQLENEVASLENENETLKKKNLHKKDLIAYLEKEIANLRKKIEE

SEQ ID NO: 24 - protein, 45 aa, synthetic construct
VAQLENEVASLENENETLKKKNLHKKDLIAYLEKEIANLRKKIEE

SEQ ID NO: 25 - protein, 44 aa, synthetic construct
AQLENEVASLENENETLKKKNLHKKDLIAYLEKEIANLRKKIEE

SEQ ID NO: 26 - protein, 43 aa, synthetic construct
QLENEVASLENENETLKKKNLHKKDLIAYLEKEIANLRKKIEE

SEQ ID NO: 27 - protein, 42 aa, synthetic construct
LENEVASLENENETLKKKNLHKKDLIAYLEKEIANLRKKIEE

SEQ ID NO: 28 - protein, 44 aa, synthetic construct
ENEVASLENENETLKKKNLHKKDLIAYLEKEIANLRKKIEEAND

SEQ ID NO: 29 - protein, 40 aa, synthetic construct
NEVASLENENETLKKKNLHKKDLIAYLEKEIANLRKKIEE

SEQ ID NO: 30 - protein, 39 aa, synthetic construct
EVASLENENETLKKKNLHKKDLIAYLEKEIANLRKKIEE

SEQ ID NO: 31 - protein, 38 aa, synthetic construct
VASLENENETLKKKNLHKKDLIAYLEKEIANLRKKIEE

SEQ ID NO: 32 - protein, 37 aa, synthetic construct
ASLENENETLKKKNLHKKDLIAYLEKEIANLRKKIEE

SEQ ID NO: 33 - protein, 36 aa, synthetic construct
SLENENETLKKKNLHKKDLIAYLEKEIANLRKKIEE

SEQ ID NO: 34 - protein, 35 aa, synthetic construct
LENENETLKKKNLHKKDLIAYLEKEIANLRKKIEE

SEQ ID NO: 35 - protein, 34 aa, synthetic construct
ENENETLKKKNLHKKDLIAYLEKEIANLRKKIEE

SEQ ID NO: 36 - protein, 36 aa, synthetic construct
NENETLKKKNLHKKDLIAYLEKEIANLRKKIEEAND

SEQ ID NO: 37 - protein, 46 aa, synthetic construct
NLVAQLENEVASLENENETLKKKNLHKKDLIAYLEKEIANLRKKIE

SEQ ID NO: 38 - protein, 45 aa, synthetic construct
NLVAQLENEVASLENENETLKKKNLHKKDLIAYLEKEIANLRKKI

SEQ ID NO: 39 - protein, 44 aa, synthetic construct
NLVAQLENEVASLENENETLKKKNLHKKDLIAYLEKEIANLRKK

SEQ ID NO: 40 - protein, 43 aa, synthetic construct
NLVAQLENEVASLENENETLKKKNLHKKDLIAYLEKEIANLRK

SEQ ID NO: 41 - protein, 42 aa, synthetic construct
NLVAQLENEVASLENENETLKKKNLHKKDLIAYLEKEIANLR

SEQ ID NO: 42 - protein, 41 aa, synthetic construct
NLVAQLENEVASLENENETLKKKNLHKKDLIAYLEKEIANL

SEQ ID NO: 43 - protein, 40 aa, synthetic construct
NLVAQLENEVASLENENETLKKKNLHKKDLIAYLEKEIAN

SEQ ID NO: 44 - protein, 39 aa, synthetic construct
NLVAQLENEVASLENENETLKKKNLHKKDLIAYLEKEIA

SEQ ID NO: 45 - protein, 38 aa, synthetic construct
NLVAQLENEVASLENENETLKKKNLHKKDLIAYLEKEI

SEQ ID NO: 46 - protein, 37 aa, synthetic construct
NLVAQLENEVASLENENETLKKKNLHKKDLIAYLEKE

SEQ ID NO: 47 - protein, 36 aa, synthetic construct
NLVAQLENEVASLENENETLKKKNLHKKDLIAYLEK

SEQ ID NO: 48 - protein, 35 aa, synthetic construct
NLVAQLENEVASLENENETLKKKNLHKKDLIAYLE

SEQ ID NO: 49 - protein, 34 aa, synthetic construct
NLVAQLENEVASLENENETLKKKNLHKKDLIAYL

SEQ ID NO: 50 - protein, 33 aa, synthetic construct
NLVAQLENEVASLENENETLKKKNLHKKDLIAY

SEQ ID NO: 51 - protein, 49 aa, synthetic construct
RNAYLRKKIARLKKDNLQLERDEQNLEKIIANLRDEIARLENEVASHEQ

SEQ ID NO: 52 - protein, 48 aa, synthetic construct
NAYLRKKIARLKKDNLQLERDEQNLEKIIANLRDEIARLENEVASHEQ

SEQ ID NO: 53 - protein, 47 aa, synthetic construct
AYLRKKIARLKKDNLQLERDEQNLEKIIANLRDEIARLENEVASHEQ

SEQ ID NO: 54 - protein, 46 aa, synthetic construct
YLRKKIARLKKDNLQLERDEQNLEKIIANLRDEIARLENEVASHEQ

SEQ ID NO: 55 - protein, 45 aa, synthetic construct
LRKKIARLKKDNLQLERDEQNLEKIIANLRDEIARLENEVASHEQ

SEQ ID NO: 56 - protein, 44 aa, synthetic construct
RKKIARLKKDNLQLERDEQNLEKIIANLRDEIARLENEVASHEQ

SEQ ID NO: 57 - protein, 43 aa, synthetic construct
KKIARLKKDNLQLERDEQNLEKIIANLRDEIARLENEVASHEQ

SEQ ID NO: 58 - protein, 42 aa, synthetic construct
KIARLKKDNLQLERDEQNLEKIIANLRDEIARLENEVASHEQ

SEQ ID NO: 59 - protein, 44 aa, synthetic construct
IARLKKDNLQLERDEQNLEKIIANLRDEIARLENEVASHEQAND

SEQ ID NO: 60 - protein, 43 aa, synthetic construct
ARLKKDNLQLERDEQNLEKIIANLRDEIARLENEVASHEQAND

SEQ ID NO: 61 - protein, 39 aa, synthetic construct
RLKKDNLQLERDEQNLEKIIANLRDEIARLENEVASHEQ

SEQ ID NO: 62 - protein, 38 aa, synthetic construct
LKKDNLQLERDEQNLEKIIANLRDEIARLENEVASHEQ

SEQ ID NO: 63 - protein, 37 aa, synthetic construct
KKDNLQLERDEQNLEKIIANLRDEIARLENEVASHEQ

SEQ ID NO: 64 - protein, 42 aa, synthetic construct
KDNLQLERDEQNLEKIIANLRDEIARLENEVASHEQANDAND

SEQ ID NO: 65 - protein, 49 aa, synthetic construct
ARNAYLRKKIARLKKDNLQLERDEQNLEKIIANLRDEIARLENEVASHE

SEQ ID NO: 66 - protein, 48 aa, synthetic construct
ARNAYLRKKIARLKKDNLQLERDEQNLEKIIANLRDEIARLENEVASH

SEQ ID NO: 67 - protein, 47 aa, synthetic construct
ARNAYLRKKIARLKKDNLQLERDEQNLEKIIANLRDEIARLENEVAS

SEQ ID NO: 68 - protein, 46 aa, synthetic construct
ARNAYLRKKIARLKKDNLQLERDEQNLEKIIANLRDEIARLENEVA

SEQ ID NO: 69 - protein, 45 aa, synthetic construct
ARNAYLRKKIARLKKDNLQLERDEQNLEKIIANLRDEIARLENEV

SEQ ID NO: 70 - protein, 44 aa, synthetic construct
ARNAYLRKKIARLKKDNLQLERDEQNLEKIIANLRDEIARLENE

SEQ ID NO: 71 - protein, 43 aa, synthetic construct
ARNAYLRKKIARLKKDNLQLERDEQNLEKIIANLRDEIARLEN

SEQ ID NO: 72 - protein, 42 aa, synthetic construct
ARNAYLRKKIARLKKDNLQLERDEQNLEKIIANLRDEIARLE

SEQ ID NO: 73 - protein, 41 aa, synthetic construct
ARNAYLRKKIARLKKDNLQLERDEQNLEKIIANLRDEIARL

SEQ ID NO: 74 - protein, 40 aa, synthetic construct
ARNAYLRKKIARLKKDNLQLERDEQNLEKIIANLRDEIAR

SEQ ID NO: 75 - protein, 39 aa, synthetic construct
ARNAYLRKKIARLKKDNLQLERDEQNLEKIIANLRDEIA

SEQ ID NO: 76 - protein, 38 aa, synthetic construct
ARNAYLRKKIARLKKDNLQLERDEQNLEKIIANLRDEI

SEQ ID NO: 77 - protein, 37 aa, synthetic construct
ARNAYLRKKIARLKKDNLQLERDEQNLEKIIANLRDE

SEQ ID NO: 78 - protein, 36 aa, synthetic construct
ARNAYLRKKIARLKKDNLQLERDEQNLEKIIANLRD

SEQ ID NO: 79 - protein, 41 aa, synthetic construct
EVTTLENDAAFIENENAYLEKEIARLRKEKAALRNRLAHKK

SEQ ID NO: 80 - protein, 40 aa, synthetic construct
VTTLENDAAFIENENAYLEKEIARLRKEKAALRNRLAHKK

SEQ ID NO: 81 - protein, 39 aa, synthetic construct
TTLENDAAFIENENAYLEKEIARLRKEKAALRNRLAHKK

SEQ ID NO: 82 - protein, 38 aa, synthetic construct
TLENDAAFIENENAYLEKEIARLRKEKAALRNRLAHKK

SEQ ID NO: 83 - protein, 37 aa, synthetic construct
LENDAAFIENENAYLEKEIARLRKEKAALRNRLAHKK

SEQ ID NO: 84 - protein, 36 aa, synthetic construct
ENDAAFIENENAYLEKEIARLRKEKAALRNRLAHKK

SEQ ID NO: 85 - protein, 35 aa, synthetic construct
NDAAFIENENAYLEKEIARLRKEKAALRNRLAHKK

SEQ ID NO: 86 - protein, 34 aa, synthetic construct
DAAFIENENAYLEKEIARLRKEKAALRNRLAHKK

SEQ ID NO: 87 - protein, 33 aa, synthetic construct
AAFIENENAYLEKEIARLRKEKAALRNRLAHKK

SEQ ID NO: 88 - protein, 32 aa, synthetic construct
AFIENENAYLEKEIARLRKEKAALRNRLAHKK

SEQ ID NO: 89 - protein, 31 aa, synthetic construct
FIENENAYLEKEIARLRKEKAALRNRLAHKK

SEQ ID NO: 90 - protein, 30 aa, synthetic construct
IENENAYLEKEIARLRKEKAALRNRLAHKK

SEQ ID NO: 91 - protein, 29 aa, synthetic construct
ENENAYLEKEIARLRKEKAALRNRLAHKK

SEQ ID NO: 92 - protein, 28 aa, synthetic construct
NENAYLEKEIARLRKEKAALRNRLAHKK

SEQ ID NO: 93 - protein, 41 aa, synthetic construct
NEVTTLENDAAFIENENAYLEKEIARLRKEKAALRNRLAHK

SEQ ID NO: 94 - protein, 40 aa, synthetic construct
NEVTTLENDAAFIENENAYLEKEIARLRKEKAALRNRLAH

SEQ ID NO: 95 - protein, 39 aa, synthetic construct
NEVTTLENDAAFIENENAYLEKEIARLRKEKAALRNRLA

SEQ ID NO: 96 - protein, 38 aa, synthetic construct
NEVTTLENDAAFIENENAYLEKEIARLRKEKAALRNRL

SEQ ID NO: 97 - protein, 37 aa, synthetic construct
NEVTTLENDAAFIENENAYLEKEIARLRKEKAALRNR

SEQ ID NO: 98 - protein, 36 aa, synthetic construct
NEVTTLENDAAFIENENAYLEKEIARLRKEKAALRN

SEQ ID NO: 99 - protein, 35 aa, synthetic construct
NEVTTLENDAAFIENENAYLEKEIARLRKEKAALR

SEQ ID NO: 100 - protein, 34 aa, synthetic construct
NEVTTLENDAAFIENENAYLEKEIARLRKEKAAL

SEQ ID NO: 101 - protein, 33 aa, synthetic construct
NEVTTLENDAAFIENENAYLEKEIARLRKEKAA

SEQ ID NO: 102 - protein, 32 aa, synthetic construct
NEVTTLENDAAFIENENAYLEKEIARLRKEKA

SEQ ID NO: 103 - protein, 31 aa, synthetic construct
NEVTTLENDAAFIENENAYLEKEIARLRKEK

SEQ ID NO: 104 - protein, 30 aa, synthetic construct
NEVTTLENDAAFIENENAYLEKEIARLRKE

SEQ ID NO: 105 - protein, 29 aa, synthetic construct
NEVTTLENDAAFIENENAYLEKEIARLRK

SEQ ID NO: 106 - protein, 28 aa, synthetic construct
NEVTTLENDAAFIENENAYLEKEIARLR

SEQ ID NO: 107 - protein, 53 aa, synthetic construct
KVAELKNRVAVKLNRNEQLKNKVEELKNRNAYLKNELATLENEVARLENDVAE

SEQ ID NO: 108 - protein, 52 aa, synthetic construct
VAELKNRVAVKLNRNEQLKNKVEELKNRNAYLKNELATLENEVARLENDVAE

SEQ ID NO: 109 - protein, 51 aa, synthetic construct
AELKNRVAVKLNRNEQLKNKVEELKNRNAYLKNELATLENEVARLENDVAE

SEQ ID NO: 110 - protein, 50 aa, synthetic construct
ELKNRVAVKLNRNEQLKNKVEELKNRNAYLKNELATLENEVARLENDVAE

SEQ ID NO: 111 - protein, 49 aa, synthetic construct
LKNRVAVKLNRNEQLKNKVEELKNRNAYLKNELATLENEVARLENDVAE

SEQ ID NO: 112 - protein, 48 aa, synthetic construct
KNRVAVKLNRNEQLKNKVEELKNRNAYLKNELATLENEVARLENDVAE

SEQ ID NO: 113 - protein, 47 aa, synthetic construct
NRVAVKLNRNEQLKNKVEELKNRNAYLKNELATLENEVARLENDVAE

SEQ ID NO: 114 - protein, 46 aa, synthetic construct
RVAVKLNRNEQLKNKVEELKNRNAYLKNELATLENEVARLENDVAE

SEQ ID NO: 115 - protein, 45 aa, synthetic construct
VAVKLNRNEQLKNKVEELKNRNAYLKNELATLENEVARLENDVAE

SEQ ID NO: 116 - protein, 44 aa, synthetic construct
AVKLNRNEQLKNKVEELKNRNAYLKNELATLENEVARLENDVAE

SEQ ID NO: 117 - protein, 43 aa, synthetic construct
VKLNRNEQLKNKVEELKNRNAYLKNELATLENEVARLENDVAE

SEQ ID NO: 118 - protein, 42 aa, synthetic construct
KLNRNEQLKNKVEELKNRNAYLKNELATLENEVARLENDVAE

SEQ ID NO: 119 - protein, 41 aa, synthetic construct
LNRNEQLKNKVEELKNRNAYLKNELATLENEVARLENDVAE

SEQ ID NO: 120 - protein, 40 aa, synthetic construct
NRNEQLKNKVEELKNRNAYLKNELATLENEVARLENDVAE

SEQ ID NO: 121 - protein, 53 aa, synthetic construct
QKVAELKNRVAVKLNRNEQLKNKVEELKNRNAYLKNELATLENEVARLENDVA

SEQ ID NO: 122 - protein, 52 aa, synthetic construct
QKVAELKNRVAVKLNRNEQLKNKVEELKNRNAYLKNELATLENEVARLENDV

SEQ ID NO: 123 - protein, 51 aa, synthetic construct
QKVAELKNRVAVKLNRNEQLKNKVEELKNRNAYLKNELATLENEVARLEND

SEQ ID NO: 124 - protein, 50 aa, synthetic construct
QKVAELKNRVAVKLNRNEQLKNKVEELKNRNAYLKNELATLENEVARLEN

SEQ ID NO: 125 - protein, 49 aa, synthetic construct
QKVAELKNRVAVKLNRNEQLKNKVEELKNRNAYLKNELATLENEVARLE

SEQ ID NO: 126 - protein, 48 aa, synthetic construct
QKVAELKNRVAVKLNRNEQLKNKVEELKNRNAYLKNELATLENEVARL

SEQ ID NO: 127 - protein, 47 aa, synthetic construct
QKVAELKNRVAVKLNRNEQLKNKVEELKNRNAYLKNELATLENEVAR

SEQ ID NO: 128 - protein, 46 aa, synthetic construct
QKVAELKNRVAVKLNRNEQLKNKVEELKNRNAYLKNELATLENEVA

SEQ ID NO: 129 - protein, 45 aa, synthetic construct
QKVAELKNRVAVKLNRNEQLKNKVEELKNRNAYLKNELATLENEV

SEQ ID NO: 130 - protein, 44 aa, synthetic construct
QKVAELKNRVAVKLNRNEQLKNKVEELKNRNAYLKNELATLENE

SEQ ID NO: 131 - protein, 43 aa, synthetic construct
QKVAELKNRVAVKLNRNEQLKNKVEELKNRNAYLKNELATLEN

SEQ ID NO: 132 - protein, 42 aa, synthetic construct
QKVAELKNRVAVKLNRNEQLKNKVEELKNRNAYLKNELATLE

SEQ ID NO: 133 - protein, 41 aa, synthetic construct
QKVAELKNRVAVKLNRNEQLKNKVEELKNRNAYLKNELATL

SEQ ID NO: 134 - protein, 40 aa, synthetic construct
QKVAELKNRVAVKLNRNEQLKNKVEELKNRNAYLKNELAT

SEQ ID NO: 135 - protein, 43 aa, synthetic construct
TVKELKNYIQELEERNAELKNLKEHLKFAKAELEFELAAHKFE

SEQ ID NO: 136 - protein, 42 aa, synthetic construct
VKELKNYIQELEERNAELKNLKEHLKFAKAELEFELAAHKFE

SEQ ID NO: 137 - protein, 41 aa, synthetic construct
KELKNYIQELEERNAELKNLKEHLKFAKAELEFELAAHKFE

SEQ ID NO: 138 - protein, 40 aa, synthetic construct
ELKNYIQELEERNAELKNLKEHLKFAKAELEFELAAHKFE

SEQ ID NO: 139 - protein, 39 aa, synthetic construct
LKNYIQELEERNAELKNLKEHLKFAKAELEFELAAHKFE

SEQ ID NO: 140 - protein, 38 aa, synthetic construct
KNYIQELEERNAELKNLKEHLKFAKAELEFELAAHKFE

SEQ ID NO: 141 - protein, 37 aa, synthetic construct
NYIQELEERNAELKNLKEHLKFAKAELEFELAAHKFE

SEQ ID NO: 142 - protein, 36 aa, synthetic construct
YIQELEERNAELKNLKEHLKFAKAELEFELAAHKFE

SEQ ID NO: 143 - protein, 35 aa, synthetic construct
IQELEERNAELKNLKEHLKFAKAELEFELAAHKFE

SEQ ID NO: 144 - protein, 34 aa, synthetic construct
QELEERNAELKNLKEHLKFAKAELEFELAAHKFE

SEQ ID NO: 145 - protein, 33 aa, synthetic construct
ELEERNAELKNLKEHLKFAKAELEFELAAHKFE

SEQ ID NO: 146 - protein, 32 aa, synthetic construct
LEERNAELKNLKEHLKFAKAELEFELAAHKFE

SEQ ID NO: 147 - protein, 31 aa, synthetic construct
EERNAELKNLKEHLKFAKAELEFELAAHKFE

SEQ ID NO: 148 - protein, 30 aa, synthetic construct
ERNAELKNLKEHLKFAKAELEFELAAHKFE

SEQ ID NO: 149 - protein, 43 aa, synthetic construct
NTVKELKNYIQELEERNAELKNLKEHLKFAKAELEFELAAHKF

SEQ ID NO: 150 - protein, 42 aa, synthetic construct
NTVKELKNYIQELEERNAELKNLKEHLKFAKAELEFELAAHK

SEQ ID NO: 151 - protein, 41 aa, synthetic construct
NTVKELKNYIQELEERNAELKNLKEHLKFAKAELEFELAAH

SEQ ID NO: 152 - protein, 40 aa, synthetic construct
NTVKELKNYIQELEERNAELKNLKEHLKFAKAELEFELAA

SEQ ID NO: 153 - protein, 39 aa, synthetic construct
NTVKELKNYIQELEERNAELKNLKEHLKFAKAELEFELA

SEQ ID NO: 154 - protein, 38 aa, synthetic construct
NTVKELKNYIQELEERNAELKNLKEHLKFAKAELEFEL

SEQ ID NO: 155 - protein, 37 aa, synthetic construct
NTVKELKNYIQELEERNAELKNLKEHLKFAKAELEFE

SEQ ID NO: 156 - protein, 36 aa, synthetic construct
NTVKELKNYIQELEERNAELKNLKEHLKFAKAELEF

SEQ ID NO: 157 - protein, 35 aa, synthetic construct
NTVKELKNYIQELEERNAELKNLKEHLKFAKAELE

SEQ ID NO: 158 - protein, 34 aa, synthetic construct
NTVKELKNYIQELEERNAELKNLKEHLKFAKAEL

SEQ ID NO: 159 - protein, 33 aa, synthetic construct
NTVKELKNYIQELEERNAELKNLKEHLKFAKAE

SEQ ID NO: 160 - protein, 32 aa, synthetic construct
NTVKELKNYIQELEERNAELKNLKEHLKFAKA

SEQ ID NO: 161 - protein, 31 aa, synthetic construct
NTVKELKNYIQELEERNAELKNLKEHLKFAK

SEQ ID NO: 162 - protein, 30 aa, synthetic construct
NTVKELKNYIQELEERNAELKNLKEHLKFA

SEQ ID NO: 163 - protein, 53 aa, synthetic construct
KVAQLKNRVAYKLKENAKLENIVARLENDNANLEKDIANLEKDIANLERDVAR

SEQ ID NO: 164 - protein, 52 aa, synthetic construct
VAQLKNRVAYKLKENAKLENIVARLENDNANLEKDIANLEKDIANLERDVAR

SEQ ID NO: 165 - protein, 51 aa, synthetic construct
AQLKNRVAYKLKENAKLENIVARLENDNANLEKDIANLEKDIANLERDVAR

SEQ ID NO: 166 - protein, 50 aa, synthetic construct
QLKNRVAYKLKENAKLENIVARLENDNANLEKDIANLEKDIANLERDVAR

SEQ ID NO: 167 - protein, 49 aa, synthetic construct
LKNRVAYKLKENAKLENIVARLENDNANLEKDIANLEKDIANLERDVAR

SEQ ID NO: 168 - protein, 48 aa, synthetic construct
KNRVAYKLKENAKLENIVARLENDNANLEKDIANLEKDIANLERDVAR

SEQ ID NO: 169 - protein, 47 aa, synthetic construct
NRVAYKLKENAKLENIVARLENDNANLEKDIANLEKDIANLERDVAR

SEQ ID NO: 170 - protein, 46 aa, synthetic construct
RVAYKLKENAKLENIVARLENDNANLEKDIANLEKDIANLERDVAR

SEQ ID NO: 171 - protein, 45 aa, synthetic construct
VAYKLKENAKLENIVARLENDNANLEKDIANLEKDIANLERDVAR

SEQ ID NO: 172 - protein, 44 aa, synthetic construct
AYKLKENAKLENIVARLENDNANLEKDIANLEKDIANLERDVAR

SEQ ID NO: 173 - protein, 43 aa, synthetic construct
YKLKENAKLENIVARLENDNANLEKDIANLEKDIANLERDVAR

SEQ ID NO: 174 - protein, 42 aa, synthetic construct
KLKENAKLENIVARLENDNANLEKDIANLEKDIANLERDVAR

SEQ ID NO: 175 - protein, 41 aa, synthetic construct
LKENAKLENIVARLENDNANLEKDIANLEKDIANLERDVAR

SEQ ID NO: 176 - protein, 40 aa, synthetic construct
KENAKLENIVARLENDNANLEKDIANLEKDIANLERDVAR

SEQ ID NO: 177 - protein, 53 aa, synthetic construct
QKVAQLKNRVAYKLKENAKLENIVARLENDNANLEKDIANLEKDIANLERDVA

SEQ ID NO: 178 - protein, 52 aa, synthetic construct
QKVAQLKNRVAYKLKENAKLENIVARLENDNANLEKDIANLEKDIANLERDV

SEQ ID NO: 179 - protein, 51 aa, synthetic construct
QKVAQLKNRVAYKLKENAKLENIVARLENDNANLEKDIANLEKDIANLERD

SEQ ID NO: 180 - protein, 50 aa, synthetic construct
QKVAQLKNRVAYKLKENAKLENIVARLENDNANLEKDIANLEKDIANLER

SEQ ID NO: 181 - protein, 49 aa, synthetic construct
QKVAQLKNRVAYKLKENAKLENIVARLENDNANLEKDIANLEKDIANLE

SEQ ID NO: 182 - protein, 48 aa, synthetic construct
QKVAQLKNRVAYKLKENAKLENIVARLENDNANLEKDIANLEKDIANL

SEQ ID NO: 183 - protein, 47 aa, synthetic construct
QKVAQLKNRVAYKLKENAKLENIVARLENDNANLEKDIANLEKDIAN

SEQ ID NO: 184 - protein, 46 aa, synthetic construct
QKVAQLKNRVAYKLKENAKLENIVARLENDNANLEKDIANLEKDIA

SEQ ID NO: 185 - protein, 45 aa, synthetic construct
QKVAQLKNRVAYKLKENAKLENIVARLENDNANLEKDIANLEKDI

SEQ ID NO: 186 - protein, 44 aa, synthetic construct
QKVAQLKNRVAYKLKENAKLENIVARLENDNANLEKDIANLEKD

SEQ ID NO: 187 - protein, 43 aa, synthetic construct
QKVAQLKNRVAYKLKENAKLENIVARLENDNANLEKDIANLEK

SEQ ID NO: 188 - protein, 42 aa, synthetic construct
QKVAQLKNRVAYKLKENAKLENIVARLENDNANLEKDIANLE

SEQ ID NO: 189 - protein, 41 aa, synthetic construct
QKVAQLKNRVAYKLKENAKLENIVARLENDNANLEKDIANL

SEQ ID NO: 190 - protein, 40 aa, synthetic construct
QKVAQLKNRVAYKLKENAKLENIVARLENDNANLEKDIAN

SEQ ID NO: 191 - protein, 41 aa, synthetic construct
LTDELKNKKEALRKDNAALLNELASLENEIANLEKEIAYFK

SEQ ID NO: 192 - protein, 40 aa, synthetic construct
TDELKNKKEALRKDNAALLNELASLENEIANLEKEIAYFK

SEQ ID NO: 193 - protein, 39 aa, synthetic construct
DELKNKKEALRKDNAALLNELASLENEIANLEKEIAYFK

SEQ ID NO: 194 - protein, 38 aa, synthetic construct
ELKNKKEALRKDNAALLNELASLENEIANLEKEIAYFK

SEQ ID NO: 195 - protein, 37 aa, synthetic construct
LKNKKEALRKDNAALLNELASLENEIANLEKEIAYFK

SEQ ID NO: 196 - protein, 36 aa, synthetic construct
KNKKEALRKDNAALLNELASLENEIANLEKEIAYFK

SEQ ID NO: 197 - protein, 35 aa, synthetic construct
NKKEALRKDNAALLNELASLENEIANLEKEIAYFK

SEQ ID NO: 198 - protein, 34 aa, synthetic construct
KKEALRKDNAALLNELASLENEIANLEKEIAYFK

SEQ ID NO: 199 - protein, 33 aa, synthetic construct
KEALRKDNAALLNELASLENEIANLEKEIAYFK

SEQ ID NO: 200 - protein, 32 aa, synthetic construct
EALRKDNAALLNELASLENEIANLEKEIAYFK

SEQ ID NO: 201 - protein, 31 aa, synthetic construct
ALRKDNAALLNELASLENEIANLEKEIAYFK

SEQ ID NO: 202 - protein, 30 aa, synthetic construct
LRKDNAALLNELASLENEIANLEKEIAYFK

SEQ ID NO: 203 - protein, 29 aa, synthetic construct
RKDNAALLNELASLENEIANLEKEIAYFK

SEQ ID NO: 204 - protein, 28 aa, synthetic construct
KDNAALLNELASLENEIANLEKEIAYFK

SEQ ID NO: 205 - protein, 41 aa, synthetic construct
ELTDELKNKKEALRKDNAALLNELASLENEIANLEKEIAYF

SEQ ID NO: 206 - protein, 40 aa, synthetic construct
ELTDELKNKKEALRKDNAALLNELASLENEIANLEKEIAY

SEQ ID NO: 207 - protein, 39 aa, synthetic construct
ELTDELKNKKEALRKDNAALLNELASLENEIANLEKEIA

SEQ ID NO: 208 - protein, 38 aa, synthetic construct
ELTDELKNKKEALRKDNAALLNELASLENEIANLEKEI

SEQ ID NO: 209 - protein, 37 aa, synthetic construct
ELTDELKNKKEALRKDNAALLNELASLENEIANLEKE

SEQ ID NO: 210 - protein, 36 aa, synthetic construct
ELTDELKNKKEALRKDNAALLNELASLENEIANLEK

SEQ ID NO: 211 - protein, 35 aa, synthetic construct
ELTDELKNKKEALRKDNAALLNELASLENEIANLE

SEQ ID NO: 212 - protein, 34 aa, synthetic construct
ELTDELKNKKEALRKDNAALLNELASLENEIANL

SEQ ID NO: 213 - protein, 33 aa, synthetic construct
ELTDELKNKKEALRKDNAALLNELASLENEIAN

SEQ ID NO: 214 - protein, 32 aa, synthetic construct
ELTDELKNKKEALRKDNAALLNELASLENEIA

SEQ ID NO: 215 - protein, 31 aa, synthetic construct
ELTDELKNKKEALRKDNAALLNELASLENEI

SEQ ID NO: 216 - protein, 30 aa, synthetic construct
ELTDELKNKKEALRKDNAALLNELASLENE

SEQ ID NO: 217 - protein, 29 aa, synthetic construct
ELTDELKNKKEALRKDNAALLNELASLEN

SEQ ID NO: 218 - protein, 28 aa, synthetic construct
ELTDELKNKKEALRKDNAALLNELASLE

SEQ ID NO: 219 - protein, 46 aa, synthetic construct
DLDAYEREAEKLEKKNEVLRNRLAALENELATLRQEVASMKQELQS

SEQ ID NO: 220 - protein, 45 aa, synthetic construct
LDAYEREAEKLEKKNEVLRNRLAALENELATLRQEVASMKQELQS

SEQ ID NO: 221 - protein, 44 aa, synthetic construct
DAYEREAEKLEKKNEVLRNRLAALENELATLRQEVASMKQELQS

SEQ ID NO: 222 - protein, 43 aa, synthetic construct
AYEREAEKLEKKNEVLRNRLAALENELATLRQEVASMKQELQS

SEQ ID NO: 223 - protein, 42 aa, synthetic construct
YEREAEKLEKKNEVLRNRLAALENELATLRQEVASMKQELQS

SEQ ID NO: 224 - protein, 41 aa, synthetic construct
EREAEKLEKKNEVLRNRLAALENELATLRQEVASMKQELQS

SEQ ID NO: 225 - protein, 40 aa, synthetic construct
REAEKLEKKNEVLRNRLAALENELATLRQEVASMKQELQS

SEQ ID NO: 226 - protein, 39 aa, synthetic construct
EAEKLEKKNEVLRNRLAALENELATLRQEVASMKQELQS

SEQ ID NO: 227 - protein, 38 aa, synthetic construct
AEKLEKKNEVLRNRLAALENELATLRQEVASMKQELQS

SEQ ID NO: 228 - protein, 37 aa, synthetic construct
EKLEKKNEVLRNRLAALENELATLRQEVASMKQELQS

SEQ ID NO: 229 - protein, 36 aa, synthetic construct
KLEKKNEVLRNRLAALENELATLRQEVASMKQELQS

SEQ ID NO: 230 - protein, 35 aa, synthetic construct
LEKKNEVLRNRLAALENELATLRQEVASMKQELQS

SEQ ID NO: 231 - protein, 34 aa, synthetic construct
EKKNEVLRNRLAALENELATLRQEVASMKQELQS

SEQ ID NO: 232 - protein, 33 aa, synthetic construct
KKNEVLRNRLAALENELATLRQEVASMKQELQS

SEQ ID NO: 233 - protein, 46 aa, synthetic construct
NDLDAYEREAEKLEKKNEVLRNRLAALENELATLRQEVASMKQELQ

SEQ ID NO: 234 - protein, 45 aa, synthetic construct
NDLDAYEREAEKLEKKNEVLRNRLAALENELATLRQEVASMKQEL

SEQ ID NO: 235 - protein, 44 aa, synthetic construct
NDLDAYEREAEKLEKKNEVLRNRLAALENELATLRQEVASMKQE

SEQ ID NO: 236 - protein, 43 aa, synthetic construct
NDLDAYEREAEKLEKKNEVLRNRLAALENELATLRQEVASMKQ

SEQ ID NO: 237 - protein, 42 aa, synthetic construct
NDLDAYEREAEKLEKKNEVLRNRLAALENELATLRQEVASMK

SEQ ID NO: 238 - protein, 41 aa, synthetic construct
NDLDAYEREAEKLEKKNEVLRNRLAALENELATLRQEVASM

SEQ ID NO: 239 - protein, 40 aa, synthetic construct
NDLDAYEREAEKLEKKNEVLRNRLAALENELATLRQEVAS

SEQ ID NO: 240 - protein, 39 aa, synthetic construct
NDLDAYEREAEKLEKKNEVLRNRLAALENELATLRQEVA

SEQ ID NO: 241 - protein, 38 aa, synthetic construct
NDLDAYEREAEKLEKKNEVLRNRLAALENELATLRQEV

SEQ ID NO: 242 - protein, 37 aa, synthetic construct
NDLDAYEREAEKLEKKNEVLRNRLAALENELATLRQE

SEQ ID NO: 243 - protein, 36 aa, synthetic construct
NDLDAYEREAEKLEKKNEVLRNRLAALENELATLRQ

SEQ ID NO: 244 - protein, 35 aa, synthetic construct
NDLDAYEREAEKLEKKNEVLRNRLAALENELATLR

SEQ ID NO: 245 - protein, 34 aa, synthetic construct
NDLDAYEREAEKLEKKNEVLRNRLAALENELATL

SEQ ID NO: 246 - protein, 33 aa, synthetic construct
NDLDAYEREAEKLEKKNEVLRNRLAALENELAT

SEQ ID NO: 247 - protein, 41 aa, synthetic construct
ILASLENKKEELKKLNAHLLKEIENLEKEIANLEKEIAYFK

SEQ ID NO: 248 - protein, 40 aa, synthetic construct
LASLENKKEELKKLNAHLLKEIENLEKEIANLEKEIAYFK

SEQ ID NO: 249 - protein, 39 aa, synthetic construct
ASLENKKEELKKLNAHLLKEIENLEKEIANLEKEIAYFK

SEQ ID NO: 250 - protein, 38 aa, synthetic construct
SLENKKEELKKLNAHLLKEIENLEKEIANLEKEIAYFK

SEQ ID NO: 251 - protein, 37 aa, synthetic construct
LENKKEELKKLNAHLLKEIENLEKEIANLEKEIAYFK

SEQ ID NO: 252 - protein, 36 aa, synthetic construct
ENKKEELKKLNAHLLKEIENLEKEIANLEKEIAYFK

SEQ ID NO: 253 - protein, 35 aa, synthetic construct
NKKEELKKLNAHLLKEIENLEKEIANLEKEIAYFK

SEQ ID NO: 254 - protein, 34 aa, synthetic construct
KKEELKKLNAHLLKEIENLEKEIANLEKEIAYFK

SEQ ID NO: 255 - protein, 33 aa, synthetic construct
KEELKKLNAHLLKEIENLEKEIANLEKEIAYFK

SEQ ID NO: 256 - protein, 32 aa, synthetic construct
EELKKLNAHLLKEIENLEKEIANLEKEIAYFK

SEQ ID NO: 257 - protein, 31 aa, synthetic construct
ELKKLNAHLLKEIENLEKEIANLEKEIAYFK

SEQ ID NO: 258 - protein, 30 aa, synthetic construct
LKKLNAHLLKEIENLEKEIANLEKEIAYFK

SEQ ID NO: 259 - protein, 29 aa, synthetic construct
KKLNAHLLKEIENLEKEIANLEKEIAYFK

SEQ ID NO: 260 - protein, 28 aa, synthetic construct
KLNAHLLKEIENLEKEIANLEKEIAYFK

SEQ ID NO: 261 - protein, 41 aa, synthetic construct
NILASLENKKEELKKLNAHLLKEIENLEKEIANLEKEIAYF

SEQ ID NO: 262 - protein, 40 aa, synthetic construct
NILASLENKKEELKKLNAHLLKEIENLEKEIANLEKEIAY

SEQ ID NO: 263 - protein, 39 aa, synthetic construct
NILASLENKKEELKKLNAHLLKEIENLEKEIANLEKEIA

SEQ ID NO: 264 - protein, 38 aa, synthetic construct
NILASLENKKEELKKLNAHLLKEIENLEKEIANLEKEI

SEQ ID NO: 265 - protein, 37 aa, synthetic construct
NILASLENKKEELKKLNAHLLKEIENLEKEIANLEKE

SEQ ID NO: 266 - protein, 36 aa, synthetic construct
NILASLENKKEELKKLNAHLLKEIENLEKEIANLEK

SEQ ID NO: 267 - protein, 35 aa, synthetic construct
NILASLENKKEELKKLNAHLLKEIENLEKEIANLE

SEQ ID NO: 268 - protein, 34 aa, synthetic construct
NILASLENKKEELKKLNAHLLKEIENLEKEIANL

SEQ ID NO: 269 - protein, 33 aa, synthetic construct
NILASLENKKEELKKLNAHLLKEIENLEKEIAN

SEQ ID NO: 270 - protein, 32 aa, synthetic construct
NILASLENKKEELKKLNAHLLKEIENLEKEIA

SEQ ID NO: 271 - protein, 31 aa, synthetic construct
NILASLENKKEELKKLNAHLLKEIENLEKEI

SEQ ID NO: 272 - protein, 30 aa, synthetic construct
NILASLENKKEELKKLNAHLLKEIENLEKE

SEQ ID NO: 273 - protein, 29 aa, synthetic construct
NILASLENKKEELKKLNAHLLKEIENLEK

SEQ ID NO: 274 - protein, 28 aa, synthetic construct
NILASLENKKEELKKLNAHLLKEIENLE

SEQ ID NO: 275 - protein, 41 aa, synthetic construct
EKEELKSKKAELRNRIEQLKQKREQLKQKIANLRKEIEAYK

SEQ ID NO: 276 - protein, 40 aa, synthetic construct
KEELKSKKAELRNRIEQLKQKREQLKQKIANLRKEIEAYK

SEQ ID NO: 277 - protein, 39 aa, synthetic construct
EELKSKKAELRNRIEQLKQKREQLKQKIANLRKEIEAYK

SEQ ID NO: 278 - protein, 38 aa, synthetic construct
ELKSKKAELRNRIEQLKQKREQLKQKIANLRKEIEAYK

SEQ ID NO: 279 - protein, 37 aa, synthetic construct
LKSKKAELRNRIEQLKQKREQLKQKIANLRKEIEAYK

SEQ ID NO: 280 - protein, 36 aa, synthetic construct
KSKKAELRNRIEQLKQKREQLKQKIANLRKEIEAYK

SEQ ID NO: 281 - protein, 35 aa, synthetic construct
SKKAELRNRIEQLKQKREQLKQKIANLRKEIEAYK

SEQ ID NO: 282 - protein, 34 aa, synthetic construct
KKAELRNRIEQLKQKREQLKQKIANLRKEIEAYK

SEQ ID NO: 283 - protein, 33 aa, synthetic construct
KAELRNRIEQLKQKREQLKQKIANLRKEIEAYK

SEQ ID NO: 284 - protein, 32 aa, synthetic construct
AELRNRIEQLKQKREQLKQKIANLRKEIEAYK

SEQ ID NO: 285 - protein, 31 aa, synthetic construct
ELRNRIEQLKQKREQLKQKIANLRKEIEAYK

SEQ ID NO: 286 - protein, 30 aa, synthetic construct
LRNRIEQLKQKREQLKQKIANLRKEIEAYK

SEQ ID NO: 287 - protein, 29 aa, synthetic construct
RNRIEQLKQKREQLKQKIANLRKEIEAYK

SEQ ID NO: 288 - protein, 28 aa, synthetic construct
NRIEQLKQKREQLKQKIANLRKEIEAYK

SEQ ID NO: 289 - protein, 41 aa, synthetic construct
NEKEELKSKKAELRNRIEQLKQKREQLKQKIANLRKEIEAY

SEQ ID NO: 290 - protein, 40 aa, synthetic construct
NEKEELKSKKAELRNRIEQLKQKREQLKQKIANLRKEIEA

SEQ ID NO: 291 - protein, 39 aa, synthetic construct
NEKEELKSKKAELRNRIEQLKQKREQLKQKIANLRKEIE

SEQ ID NO: 292 - protein, 38 aa, synthetic construct
NEKEELKSKKAELRNRIEQLKQKREQLKQKIANLRKEI

SEQ ID NO: 293 - protein, 37 aa, synthetic construct
NEKEELKSKKAELRNRIEQLKQKREQLKQKIANLRKE

SEQ ID NO: 294 - protein, 36 aa, synthetic construct
NEKEELKSKKAELRNRIEQLKQKREQLKQKIANLRK

SEQ ID NO: 295 - protein, 35 aa, synthetic construct
NEKEELKSKKAELRNRIEQLKQKREQLKQKIANLR

SEQ ID NO: 296 - protein, 34 aa, synthetic construct
NEKEELKSKKAELRNRIEQLKQKREQLKQKIANL

SEQ ID NO: 297 - protein, 33 aa, synthetic construct
NEKEELKSKKAELRNRIEQLKQKREQLKQKIAN

SEQ ID NO: 298 - protein, 32 aa, synthetic construct
NEKEELKSKKAELRNRIEQLKQKREQLKQKIA

SEQ ID NO: 299 - protein, 31 aa, synthetic construct
NEKEELKSKKAELRNRIEQLKQKREQLKQKI

SEQ ID NO: 300 - protein, 30 aa, synthetic construct
NEKEELKSKKAELRNRIEQLKQKREQLKQK

SEQ ID NO: 301 - protein, 29 aa, synthetic construct
NEKEELKSKKAELRNRIEQLKQKREQLKQ

SEQ ID NO: 302 - protein, 28 aa, synthetic construct
NEKEELKSKKAELRNRIEQLKQKREQLK

SEQ ID NO: 303 - protein, 40 aa, synthetic construct
IAATLENDLARLENENARLEKDIANLERDLAKLEREEAYF

SEQ ID NO: 304 - protein, 39 aa, synthetic construct
AATLENDLARLENENARLEKDIANLERDLAKLEREEAYF

SEQ ID NO: 305 - protein, 38 aa, synthetic construct
ATLENDLARLENENARLEKDIANLERDLAKLEREEAYF

SEQ ID NO: 306 - protein, 37 aa, synthetic construct
TLENDLARLENENARLEKDIANLERDLAKLEREEAYF

SEQ ID NO: 307 - protein, 36 aa, synthetic construct
LENDLARLENENARLEKDIANLERDLAKLEREEAYF

SEQ ID NO: 308 - protein, 35 aa, synthetic construct
ENDLARLENENARLEKDIANLERDLAKLEREEAYF

SEQ ID NO: 309 - protein, 34 aa, synthetic construct
NDLARLENENARLEKDIANLERDLAKLEREEAYF

SEQ ID NO: 310 - protein, 33 aa, synthetic construct
DLARLENENARLEKDIANLERDLAKLEREEAYF

SEQ ID NO: 311 - protein, 32 aa, synthetic construct
LARLENENARLEKDIANLERDLAKLEREEAYF

SEQ ID NO: 312 - protein, 31 aa, synthetic construct
ARLENENARLEKDIANLERDLAKLEREEAYF

SEQ ID NO: 313 - protein, 30 aa, synthetic construct
RLENENARLEKDIANLERDLAKLEREEAYF

SEQ ID NO: 314 - protein, 29 aa, synthetic construct
LENENARLEKDIANLERDLAKLEREEAYF

SEQ ID NO: 315 - protein, 28 aa, synthetic construct
ENENARLEKDIANLERDLAKLEREEAYF

SEQ ID NO: 316 - protein, 27 aa, synthetic construct
NENARLEKDIANLERDLAKLEREEAYF

SEQ ID NO: 317 - protein, 40 aa, synthetic construct
SIAATLENDLARLENENARLEKDIANLERDLAKLEREEAY

SEQ ID NO: 318 - protein, 39 aa, synthetic construct
SIAATLENDLARLENENARLEKDIANLERDLAKLEREEA

SEQ ID NO: 319 - protein, 38 aa, synthetic construct
SIAATLENDLARLENENARLEKDIANLERDLAKLEREE

SEQ ID NO: 320 - protein, 37 aa, synthetic construct
SIAATLENDLARLENENARLEKDIANLERDLAKLERE

SEQ ID NO: 321 - protein, 36 aa, synthetic construct
SIAATLENDLARLENENARLEKDIANLERDLAKLER

SEQ ID NO: 322 - protein, 35 aa, synthetic construct
SIAATLENDLARLENENARLEKDIANLERDLAKLE

SEQ ID NO: 323 - protein, 34 aa, synthetic construct
SIAATLENDLARLENENARLEKDIANLERDLAKL

SEQ ID NO: 324 - protein, 33 aa, synthetic construct
SIAATLENDLARLENENARLEKDIANLERDLAK

SEQ ID NO: 325 - protein, 32 aa, synthetic construct
SIAATLENDLARLENENARLEKDIANLERDLA

SEQ ID NO: 326 - protein, 31 aa, synthetic construct
SIAATLENDLARLENENARLEKDIANLERDL

SEQ ID NO: 327 - protein, 30 aa, synthetic construct
SIAATLENDLARLENENARLEKDIANLERD

SEQ ID NO: 328 - protein, 29 aa, synthetic construct
SIAATLENDLARLENENARLEKDIANLER

SEQ ID NO: 329 - protein, 28 aa, synthetic construct
SIAATLENDLARLENENARLEKDIANLE

SEQ ID NO: 330 - protein, 27 aa, synthetic construct
SIAATLENDLARLENENARLEKDIANL

SEQ ID NO: 331 - protein, 44 aa, synthetic construct
ELESLENKKEELKNRNEELKQKREQLKQKLAALRNKLDAYKNRL

SEQ ID NO: 332 - protein, 46 aa, synthetic construct
LESLENKKEELKNRNEELKQKREQLKQKLAALRNKLDAYKNRLAND

SEQ ID NO: 333 - protein, 42 aa, synthetic construct
ESLENKKEELKNRNEELKQKREQLKQKLAALRNKLDAYKNRL

SEQ ID NO: 334 - protein, 41 aa, synthetic construct
SLENKKEELKNRNEELKQKREQLKQKLAALRNKLDAYKNRL

SEQ ID NO: 335 - protein, 40 aa, synthetic construct
LENKKEELKNRNEELKQKREQLKQKLAALRNKLDAYKNRL

SEQ ID NO: 336 - protein, 39 aa, synthetic construct
ENKKEELKNRNEELKQKREQLKQKLAALRNKLDAYKNRL

SEQ ID NO: 337 - protein, 41 aa, synthetic construct
NKKEELKNRNEELKQKREQLKQKLAALRNKLDAYKNRLAND

SEQ ID NO: 338 - protein, 37 aa, synthetic construct
KKEELKNRNEELKQKREQLKQKLAALRNKLDAYKNRL

SEQ ID NO: 339 - protein, 36 aa, synthetic construct
KEELKNRNEELKQKREQLKQKLAALRNKLDAYKNRL

SEQ ID NO: 340 - protein, 35 aa, synthetic construct
EELKNRNEELKQKREQLKQKLAALRNKLDAYKNRL

SEQ ID NO: 341 - protein, 34 aa, synthetic construct
ELKNRNEELKQKREQLKQKLAALRNKLDAYKNRL

SEQ ID NO: 342 - protein, 33 aa, synthetic construct
LKNRNEELKQKREQLKQKLAALRNKLDAYKNRL

SEQ ID NO: 343 - protein, 32 aa, synthetic construct
KNRNEELKQKREQLKQKLAALRNKLDAYKNRL

SEQ ID NO: 344 - protein, 31 aa, synthetic construct
NRNEELKQKREQLKQKLAALRNKLDAYKNRL

SEQ ID NO: 345 - protein, 44 aa, synthetic construct
NELESLENKKEELKNRNEELKQKREQLKQKLAALRNKLDAYKNR

SEQ ID NO: 346 - protein, 43 aa, synthetic construct
NELESLENKKEELKNRNEELKQKREQLKQKLAALRNKLDAYKN

SEQ ID NO: 347 - protein, 42 aa, synthetic construct
NELESLENKKEELKNRNEELKQKREQLKQKLAALRNKLDAYK

SEQ ID NO: 348 - protein, 41 aa, synthetic construct
NELESLENKKEELKNRNEELKQKREQLKQKLAALRNKLDAY

SEQ ID NO: 349 - protein, 40 aa, synthetic construct
NELESLENKKEELKNRNEELKQKREQLKQKLAALRNKLDA

SEQ ID NO: 350 - protein, 39 aa, synthetic construct
NELESLENKKEELKNRNEELKQKREQLKQKLAALRNKLD

SEQ ID NO: 351 - protein, 38 aa, synthetic construct
NELESLENKKEELKNRNEELKQKREQLKQKLAALRNKL

SEQ ID NO: 352 - protein, 37 aa, synthetic construct
NELESLENKKEELKNRNEELKQKREQLKQKLAALRNK

SEQ ID NO: 353 - protein, 36 aa, synthetic construct
NELESLENKKEELKNRNEELKQKREQLKQKLAALRN

SEQ ID NO: 354 - protein, 35 aa, synthetic construct
NELESLENKKEELKNRNEELKQKREQLKQKLAALR

SEQ ID NO: 355 - protein, 34 aa, synthetic construct
NELESLENKKEELKNRNEELKQKREQLKQKLAAL

SEQ ID NO: 356 - protein, 33 aa, synthetic construct
NELESLENKKEELKNRNEELKQKREQLKQKLAA

SEQ ID NO: 357 - protein, 32 aa, synthetic construct
NELESLENKKEELKNRNEELKQKREQLKQKLA

SEQ ID NO: 358 - protein, 31 aa, synthetic construct
NELESLENKKEELKNRNEELKQKREQLKQKL

SEQ ID NO: 359 - protein, 43 aa, synthetic construct
TVEELLRAIQELEKRNAELKNRKEELKNLVAHLRQELAAHKYE

SEQ ID NO: 360 - protein, 42 aa, synthetic construct
VEELLRAIQELEKRNAELKNRKEELKNLVAHLRQELAAHKYE

SEQ ID NO: 361 - protein, 41 aa, synthetic construct
EELLRAIQELEKRNAELKNRKEELKNLVAHLRQELAAHKYE

SEQ ID NO: 362 - protein, 40 aa, synthetic construct
ELLRAIQELEKRNAELKNRKEELKNLVAHLRQELAAHKYE

SEQ ID NO: 363 - protein, 39 aa, synthetic construct
LLRAIQELEKRNAELKNRKEELKNLVAHLRQELAAHKYE

SEQ ID NO: 364 - protein, 38 aa, synthetic construct
LRAIQELEKRNAELKNRKEELKNLVAHLRQELAAHKYE

SEQ ID NO: 365 - protein, 37 aa, synthetic construct
RAIQELEKRNAELKNRKEELKNLVAHLRQELAAHKYE

SEQ ID NO: 366 - protein, 36 aa, synthetic construct
AIQELEKRNAELKNRKEELKNLVAHLRQELAAHKYE

SEQ ID NO: 367 - protein, 35 aa, synthetic construct
IQELEKRNAELKNRKEELKNLVAHLRQELAAHKYE

SEQ ID NO: 368 - protein, 34 aa, synthetic construct
QELEKRNAELKNRKEELKNLVAHLRQELAAHKYE

SEQ ID NO: 369 - protein, 33 aa, synthetic construct
ELEKRNAELKNRKEELKNLVAHLRQELAAHKYE

SEQ ID NO: 370 - protein, 32 aa, synthetic construct
LEKRNAELKNRKEELKNLVAHLRQELAAHKYE

SEQ ID NO: 371 - protein, 31 aa, synthetic construct
EKRNAELKNRKEELKNLVAHLRQELAAHKYE

SEQ ID NO: 372 - protein, 30 aa, synthetic construct
KRNAELKNRKEELKNLVAHLRQELAAHKYE

SEQ ID NO: 373 - protein, 43 aa, synthetic construct
STVEELLRAIQELEKRNAELKNRKEELKNLVAHLRQELAAHKY

SEQ ID NO: 374 - protein, 42 aa, synthetic construct
STVEELLRAIQELEKRNAELKNRKEELKNLVAHLRQELAAHK

SEQ ID NO: 375 - protein, 41 aa, synthetic construct
STVEELLRAIQELEKRNAELKNRKEELKNLVAHLRQELAAH

SEQ ID NO: 376 - protein, 40 aa, synthetic construct
STVEELLRAIQELEKRNAELKNRKEELKNLVAHLRQELAA

SEQ ID NO: 377 - protein, 39 aa, synthetic construct
STVEELLRAIQELEKRNAELKNRKEELKNLVAHLRQELA

SEQ ID NO: 378 - protein, 38 aa, synthetic construct
STVEELLRAIQELEKRNAELKNRKEELKNLVAHLRQEL

SEQ ID NO: 379 - protein, 37 aa, synthetic construct
STVEELLRAIQELEKRNAELKNRKEELKNLVAHLRQE

SEQ ID NO: 380 - protein, 36 aa, synthetic construct
STVEELLRAIQELEKRNAELKNRKEELKNLVAHLRQ

SEQ ID NO: 381 - protein, 35 aa, synthetic construct
STVEELLRAIQELEKRNAELKNRKEELKNLVAHLR

SEQ ID NO: 382 - protein, 34 aa, synthetic construct
STVEELLRAIQELEKRNAELKNRKEELKNLVAHL

SEQ ID NO: 383 - protein, 33 aa, synthetic construct
STVEELLRAIQELEKRNAELKNRKEELKNLVAH

SEQ ID NO: 384 - protein, 32 aa, synthetic construct
STVEELLRAIQELEKRNAELKNRKEELKNLVA

SEQ ID NO: 385 - protein, 31 aa, synthetic construct
STVEELLRAIQELEKRNAELKNRKEELKNLV

SEQ ID NO: 386 - protein, 30 aa, synthetic construct
STVEELLRAIQELEKRNAELKNRKEELKNL

SEQ ID NO: 387 - protein, 41 aa, synthetic construct
EVAQLENDVAVIENENAYLEKEIARLRKEIAALRDRLAHKK

SEQ ID NO: 388 - protein, 40 aa, synthetic construct
VAQLENDVAVIENENAYLEKEIARLRKEIAALRDRLAHKK

SEQ ID NO: 389 - protein, 39 aa, synthetic construct
AQLENDVAVIENENAYLEKEIARLRKEIAALRDRLAHKK

SEQ ID NO: 390 - protein, 38 aa, synthetic construct
QLENDVAVIENENAYLEKEIARLRKEIAALRDRLAHKK

SEQ ID NO: 391 - protein, 37 aa, synthetic construct
LENDVAVIENENAYLEKEIARLRKEIAALRDRLAHKK

SEQ ID NO: 392 - protein, 36 aa, synthetic construct
ENDVAVIENENAYLEKEIARLRKEIAALRDRLAHKK

SEQ ID NO: 393 - protein, 35 aa, synthetic construct
NDVAVIENENAYLEKEIARLRKEIAALRDRLAHKK

SEQ ID NO: 394 - protein, 34 aa, synthetic construct
DVAVIENENAYLEKEIARLRKEIAALRDRLAHKK

SEQ ID NO: 395 - protein, 33 aa, synthetic construct
VAVIENENAYLEKEIARLRKEIAALRDRLAHKK

SEQ ID NO: 396 - protein, 32 aa, synthetic construct
AVIENENAYLEKEIARLRKEIAALRDRLAHKK

SEQ ID NO: 397 - protein, 31 aa, synthetic construct
VIENENAYLEKEIARLRKEIAALRDRLAHKK

SEQ ID NO: 398 - protein, 30 aa, synthetic construct
IENENAYLEKEIARLRKEIAALRDRLAHKK

SEQ ID NO: 399 - protein, 29 aa, synthetic construct
ENENAYLEKEIARLRKEIAALRDRLAHKK

SEQ ID NO: 400 - protein, 28 aa, synthetic construct
NENAYLEKEIARLRKEIAALRDRLAHKK

SEQ ID NO: 401 - protein, 41 aa, synthetic construct
NEVAQLENDVAVIENENAYLEKEIARLRKEIAALRDRLAHK

SEQ ID NO: 402 - protein, 40 aa, synthetic construct
NEVAQLENDVAVIENENAYLEKEIARLRKEIAALRDRLAH

SEQ ID NO: 403 - protein, 39 aa, synthetic construct
NEVAQLENDVAVIENENAYLEKEIARLRKEIAALRDRLA

SEQ ID NO: 404 - protein, 38 aa, synthetic construct
NEVAQLENDVAVIENENAYLEKEIARLRKEIAALRDRL

SEQ ID NO: 405 - protein, 37 aa, synthetic construct
NEVAQLENDVAVIENENAYLEKEIARLRKEIAALRDR

SEQ ID NO: 406 - protein, 36 aa, synthetic construct
NEVAQLENDVAVIENENAYLEKEIARLRKEIAALRD

SEQ ID NO: 407 - protein, 35 aa, synthetic construct
NEVAQLENDVAVIENENAYLEKEIARLRKEIAALR

SEQ ID NO: 408 - protein, 33 aa, synthetic construct
NEVAQLENDVAVIENENAYLEKEIARLRKEIAA

SEQ ID NO: 409 - protein, 32 aa, synthetic construct
NEVAQLENDVAVIENENAYLEKEIARLRKEIA

SEQ ID NO: 410 - protein, 31 aa, synthetic construct
NEVAQLENDVAVIENENAYLEKEIARLRKEI

SEQ ID NO: 411 - protein, 30 aa, synthetic construct
NEVAQLENDVAVIENENAYLEKEIARLRKE

SEQ ID NO: 412 - protein, 29 aa, synthetic construct
NEVAQLENDVAVIENENAYLEKEIARLRK

SEQ ID NO: 413 - protein, 28 aa, synthetic construct
NEVAQLENDVAVIENENAYLEKEIARLR

SEQ ID NO: 414 - protein, 27 aa, synthetic construct
NEVAQLENDVAVIENENAYLEKEIARL

SEQ ID NO: 415 - protein, 10 aa, synthetic construct
NATETVYPES